European Patent Application EP 4 790 145 A2, published August 12, 2026. Title: GENERATING CAPTURE PROBES FOR SPATIAL ANALYSIS. Applicant: 10x Genomics, Inc. Application US 19/315,008, filed August 29, 2025. The sequence listing filed with the application follows.

SEQUENCE LISTING (12 sequences)

SEQ ID NO: 1 - protein, 16 aa, synthetic construct
  REGION 1..16: note = Synthetic Trademark of PURAMATRIX polypeptide sequence
RADARADARADARADA

SEQ ID NO: 2 - protein, 16 aa, synthetic construct
  REGION 1..16: note = Synthetic EAK16 polypeptide sequence
AEAEAKAKAEAEAKAK

SEQ ID NO: 3 - protein, 12 aa, synthetic construct
  REGION 1..12: note = Synthetic KLD12 polypeptide sequence
KLDLKLDLKLDL

SEQ ID NO: 4 - DNA, 18 bp, synthetic construct
  source 1..18: mol_type = other DNA
gaggaattcccagtaagt

SEQ ID NO: 5 - DNA, 18 bp, synthetic construct
  source 1..18: mol_type = other DNA
gagattgagcaataacag

SEQ ID NO: 6 - DNA, 18 bp, synthetic construct
  source 1..18: mol_type = other DNA
gtagttccgaccataaac

SEQ ID NO: 7 - DNA, 18 bp, synthetic construct
  source 1..18: mol_type = other DNA
ggtgactctagataacct

SEQ ID NO: 8 - RNA, 35 nt, unidentified
  misc_feature 1..35: note = Analyte poly(A) tail from biological sample
  source 1..35: mol_type = unassigned RNA
aaaaaaaaaaannnnnnnnnnnnnnnnnnnnnnnn

SEQ ID NO: 9 - DNA, 68 bp, synthetic construct
  misc_feature 1..68: note = Capture Probe
  source 1..68: mol_type = other DNA
  variation 1..12: note = t=u
ttttttttttttctacacgactcttccgatctacgtacgtacgtacgtnnnnnnnnnnnngcggcccg

SEQ ID NO: 10 - DNA, 18 bp, synthetic construct
  misc_feature 1..18: note = Splint Oligonucleotide
  source 1..18: mol_type = other DNA
aaaaaaaaaacgggccgc

SEQ ID NO: 11 - DNA, 27 bp, synthetic construct
  misc_feature 1..27: note = Capture domain poly(T) sequence
  source 1..27: mol_type = other DNA
ttttttttttttttttttttttttttt

SEQ ID NO: 12 - DNA, 62 bp, synthetic construct
  misc_feature 1..62: note = Capture probe 2
  source 1..62: mol_type = other DNA
tttttctacacgacgctcttccgatctacgtacgtacgtacgtnnnnnnnnnnnncgctacg